European Patent Specification EP 3 882 355 B1, published December 20, 2023. Title: DIAGNOSTIC MARKERS FOR TREATING CELL PROLIFERATIVE DISORDERS WITH TELOMERASE INHIBITORS. Applicant: Geron Corporation Bassett, Ekaterina Burington, Bart Wang, Hui Eng, Kevin. Application EP 13858528.6. The sequence listing filed with the application follows.

SEQUENCE LISTING (10 sequences)

SEQ ID NO: 1 - RNA, 554 nt, Homo sapiens
ggguugcggagggugggccugggaggggugguggccauuuuuugucuaacccuaacugagaagggcguaggcgccgugcuuuugcuccccgcgcgcuguuuuucucgcugacuuucagcgggcggaaaagccucggccugccgccuuccaccguucauucuagagcaaacaaaaaaugucagcugcuggcccguucgccucccggggaccugcggcgggucgccugcccagcccccgaaccccgccuggagccgcggucggcccggggcuucuccggaggcacccacugccaccgcgaagaguugggcucugucagccgcgggucucucgggggcgagggcgagguucaccguuucaggccgcaggaagaggaacggagcgagucccgccgcggcgcgauucccugagcugugggacgugcacccaggacucggcucacacaugcaguucgcuuuccuguugguggggggaacgccgaucgugcgcauccgucaccccucgccggcagugggggcuugugaacccccaaaccugacugacugggccagugugcu

SEQ ID NO: 2 - RNA, 11 nt, Artificial sequence
  hTR template inhibitor
cuaacccuaac

SEQ ID NO: 3 - DNA, 13 bp, Artificial sequence
  hTR template inhibitor
tagggttagacaa

SEQ ID NO: 4 - DNA, 40 bp, Artificial sequence
  primer for telomere amplification
acactaaggtttgggtttgggtttgggtttgggttagtgt

SEQ ID NO: 5 - DNA, 42 bp, Artificial sequence
  primer for telomere amplification
tgttaggtatccctatccctatccctatccctatccctaaca

SEQ ID NO: 6 - DNA, 23 bp, Artificial sequence
  primer for telomere amplification
cagcaagtgggaaggtgtaatcc

SEQ ID NO: 7 - DNA, 28 bp, Artificial sequence
  primer for telomere amplification
cccattctatcatcatcaacgggtacaa

SEQ ID NO: 8 - DNA, 18 bp, Artificial sequence
  telomere probe
ccctaaccctaaccctaa

SEQ ID NO: 9 - DNA, 84 bp, Artificial sequence
  standard for telomere length double stranded template
ttagggttagggttagggttagggttagggttagggttagggttagggttagggttagggttagggttagggttagggttaggg

SEQ ID NO: 10 - DNA, 84 bp, Artificial sequence
  standard for single copy gene double stranded template
cttttcagcaagtgggaaggtgtaatccgtctccacagacaaggccaggactcgtttgtacccgttgatgatagaatggggtac